European Patent Application EP 4 741 417 A1, published May 13, 2026. Title: 一种角蛋白CF2、制法和其药物组合物与用途. Applicant: 中国医学科学院药物研究所. The sequence listing filed with the application follows.

SEQUENCE LISTING (2 sequences)

SEQ ID NO: 1 - protein, 478 aa, unidentified
MTTYSRQFTSSSSLKGSCGIGGGSSRISSVLGGGSYRAPSAYGGGLSVSSRYSSGGACGLGGGYGGGFSSSSSFGGALGSSYGGGYGGGLGGGLGGGFGGGFGGGLGGGFGGGDGLLVGSEKVTMQNLNDRLASYLDKVRALEEANADLEVKIRDWYQKQRPAEIKDYSPYFKTIEDLRNKILTATVDNANVVLQIDNARLAADDFRTKYETELNLRLSVEADINGLRRVLDELTLARTDLEMQIESLKEELAYLRKNHEEEMNSLRGQVGGDVNVEMDAAPGVDLSRILNEMRDQYEKIAEKNRKDAEDWFFSKTEELNREVATNSELVQSGKSEISELRRTVQNLEIELQSQLSMKASLENSLEETKGRYCMQLAQIQELISSVEEQLAQLRCEMEQQNQEYKILLDVKTRLEQEIATYRRLLEGEDAHLSSSQFSSGSQSSRDVTSSSRQIRTKVMDVHDGKVVSTHEQVLRTKN

SEQ ID NO: 2 - DNA, 1434 bp, unidentified
  source 1..1434: mol_type = other DNA
atgaccacctatagccgccagtttaccagcagcagcagcctgaaaggcagctgcggcattggcggcggttcatcacgcattagcagcgtgttaggcggcggcagctatcgtgcgccttcagcgtatggtggtggcttaagcgttagcagccgttatagcagcggcggcgcgtgtggtttaggcggcggttatggtggtggctttagcagcagcagcagctttggcggcgccctgggtagcagctatggtggcggttatggcggcggtttaggtggtggtttaggtggcggctttggtggcggctttggcggcggattaggtggtggttttggtggtggcgatggcttattagtgggcagcgaaaaagtgaccatgcagaacctgaacgatcgcctggcgagctatctggataaagtgcgtgcgttagaagaagcgaacgcggatttagaagtgaaaattcgcgattggtatcagaaacagcgcccggcggaaattaaagattatagcccgtattttaagaccatcgaggatctgcgcaacaagattctgaccgcgaccgtggataacgcgaacgtggtgctgcagattgataacgcccgcctggcggcggatgattttcgcaccaaatatgaaaccgaactgaacctgcgcctgagcgtggaagcggatattaacggcctgcgccgcgtgctggatgaactgaccttagcgcgtaccgatctggaaatgcagattgaaagcctgaaagaagaactggcgtatctgcgcaaaaaccatgaagaagaaatgaacagcctgcgcggccaggtgggcggtgatgttaatgttgaaatggatgcggcgccgggcgttgatctgagccgcattttaaatgaaatgcgcgatcagtatgagaaaattgcggagaaaaaccgcaaagacgcggaagattggttctttagcaaaaccgaagaactgaaccgcgaagtggcgaccaacagcgaactggtgcagagcggcaaaagcgaaattagcgaactgcgccgcaccgtgcagaacctggaaattgaactgcagagccagctgagcatgaaagcgagcctggaaaacagcctggaagaaaccaaaggccgctattgcatgcagctggcgcagattcaggaactgattagcagcgtggaagaacagctggcgcagctgcgctgtgaaatggaacagcagaaccaggaatataaaattctgctggatgtgaaaacccgcctggaacaggaaattgcgacctatcgccgcctgctggaaggcgaagatgcgcatttaagcagcagccagtttagcagcggcagccagagcagccgcgatgtgaccagcagcagccgtcaaattcgcaccaaagtgatggatgtgcatgatggcaaagtggtgagcacccatgaacaggtgctgcgcaccaaaaac